European Patent Application EP 4 215 611 A1, published July 26, 2023. Title: Modification of the genome of a filamentous fungus. Applicant: BRAIN Biotech AG. The sequence listing filed with the application follows.

SEQUENCE LISTING (21 sequences)

SEQ ID NO: 1 - protein, 1231 aa, Artificial Sequence
  BEC85 AA Sequence
MKSFENSCQISKTLRFGATLKEDKKKCKSHLELQEFVDISYKTLKSSATIAESLNEIELVKKCERCYSEIIKFHEAWGQIYCRTNQIAVYKDWYRQLARKARFDVGDQNSQLITLSSLSSKHNVYQGLKRSQHITNYWKDNIARQKSFLKDFSQQLKQYKRALENSDKAHTKPNLINFNKTFSILANLVNEIVIPLSNGAISFPNISKLEDGEESRHLIEFALNDYSDLVGSIGELKDAIATNGGYTPFAKVTLNHYTAEQKPHVFKNDIDAKIRELKLIELVEKLKNKTSKQIEEYFSKFDKFKIYDDRNISVIIRTQCFKYKPIPFLVKHELAKYIAEDEDAVLKVLDAIGATRSPAHDYAHNEDVFDLNHYPIKVAFDYAWEQLANSLYTTVTFPKEQCEKYLKDVFDCEVSKEPVFKFYADLLYIRKNLAVLEHKNNLPSNQEEFICKINNTFENIVLPYKISQFETYKKDILAWINDGRGHEKYTDAKQQLGFIRGGLKGRIKAQKMFRKDKYGKIKSYYENPYTKLTNEFKQISSTYGKTFAELRDKFKEKNNITKITHFGIIIEDKNRDRYLLANGLQHEQINHVSTILNKLDKSSEFITYQVKSLTSKTLIKLIKNHTTKKGAISPYADFHTSKTGFNKNEIEKNWDNYKREQVLVEYVKDCLTDSTMAKNQNWAEFGWNFEKCNSYEDIEHEIDQKSYILQKHTISKQSIASLVEGGCLLLPIINQDITSKERKDKNQFSKDWKQIFEGSKEFRLHPEFAVSYRTPIEGYPVQKRYGRLQFVCAFNCEIIPQNGEFINLKKQIENFNDEDAQKEAVEEFNKKVNHALSDKEYVVIGIDRGLKQLATLCVLDKRGKILGDFEIYKKEFVRAEKRSESHWEHTQAETRHILDLSNLRVETTIEGKKVLVDQSLTLVKKNRDTPDEEATEENKQKIKLKQLSYIRKLQHKMQTNEQDVLDLINNEPSDEEFKKRIEGLISSFGEGQKYADLPINTMREMISDLQGVIARGNNQTEKNKIIELDAADNLKQGIVANMIGIVNYIFAKYSYKAYISLEDLSRAYGGAKSGYDGRYLPSTSQDEDVDFKEQQNQMLAGLGTYQFFEMQLLKKLQKIQSDNTVLRFVPAFRSADNYRNILRLEETKYKSKPFGVVHFIDPKFTSKKCPVCSKTNVYRDKDDILVCKECGFRSDSQLKERENNIHYIHNGDDNGAYHIALKSVENLIQMK

SEQ ID NO: 2 - protein, 1231 aa, Artificial Sequence
  BEC67 AA Sequence
MKSFENSCQISKTLRFGATLKEDKKKCKSHLELQEFVDISYKTLKSSATIAESLNEIELVKKCERCYSEIIKFHEAWGQIYCRTNQIAVYKDWYRQLARKARFDVGDQNSQLITLSSLSSKHNVYQGLKRSQHITNYWKDNIARQKSFLKDFSQQLKQYKRALENSDKAHTKPNLINFNKTFSILANLVNEIVIPLSNGAISFPNISKLEDGEESRHLIEFALNDYSDLVGSIGELKDAIATNGGYTPFAKVTLNHYTAEQKPHVFKNDIDAKIRELKLIELVEKLKNKTSKQIEEYFSKFDKFKIYDDRNISVIIRTQCFKYKPIPFLVKHELAKYIAEDEDAVLKVLDAIGATRSPAHDYAHNEDVFDLNHYPIKVAFDYAWEQLANSLYTTVTFPKEQCEKYLKDVFDCEVSKEPVFKFYADLLYIRKNLAVLEHKNNLPSNQEEFICKINNTFENIVLPYKISQFETYKKDILAWINDGRGHEKYTDSKRELGFIRGGLKGRIKAQKMFRKDKYGKIKSYYENPYTKLTEEFKNLAITYGKTFAELRDKFKEKNNITKITHFGIIIEDKNRDRYLLANGLQHEQINHVSTILNKLDKSSEFITYQVKSLTSKTLIKLIKNHTTKKGAISPYADFHTSKTGFNKNEIEKNWDNYKREQVLVEYVKDCLTDSTMAKNQNWAEFGWDLESCNSYEDIEHEIDQKSYILQKHTISKQSIASLVEGGCLLLPIINQDITSKERKDKNQFSKDWKQIFEGSKEFRLHPEFAVSYRTPIEGYPVQKRYGRLQFVCAFNCEIIPQNGEFINLKKQIENFNDEDAQKEAVEEFNKKVNHALSDKEYVVIGIDRGLKQLATLCVLDKRGKILGDFEIYKKEFVRAEKRSESHWEHTQAETRHILDLSNLRVETTIEGKKVLVDQSLTLVKKNRDTPDEEATEENKQKIKLKQLSYIRKLQHKMQTNEQDVLDLINNEPSDEEFKKRIEGLISSFGEGQKYADLPINTMREMISDLQGVIARGNNQTEKNKIIELDAADNLKQGIVANMIGIVNYIFAKYSYKAYISLEDLSRAYGGAKSGYDGRYLPSTSQDEDVDFKEQQNQMLAGLGTYQFFEMQLLKKLQKIQSDNTVLRFVPAFRSADNYRNILRLEETKYKSKPFGVVHFIDPKFTSKKCPVCSKTNVYRDKDDILVCKECGFRSDSQLKERENNIHYIHNGDDNGAYHIALKSVENLIQMK

SEQ ID NO: 3 - protein, 1231 aa, Artificial Sequence
  BEC10 AA Sequence
MKSFENSCQISKTLRFGATLKEDKKKCKSHLELQEFVDISYKTLKSSATIAESLNEIELVKKCERCYSEIIKFHEAWGQIYCRTNQIAVYKDWYRQLARKARFDVGDQNSQLITLSSLSSKHNVYQGLKRSQHITNYWKDNIARQKSFLKDFSQQLKQYKRALENSDKAHTKPNLINFNKTFSILANLVNEIVIPLSNGAISFPNISKLEDGEESRHLIEFALNDYSDLVGSIGELKDAIATNGGYTPFAKVTLNHYTAEQKPHVFKNDIDAKIRELKLIELVEKLKNKTSKQIEEYFSKFDKFKIYDDRNISVIIRTQCFKYKPIPFLVKHELAKYIAEDEDAVLKVLDAIGATRSPAHDYAHNEDVFDLNHYPIKVAFDYAWEQLANGVYTTVTFPKEQCEKYLKDVFDCEVSKEPVFKFYADLLYIRKNLAVLEHKNNLPSNQEEFICKINNTFENIVLPYKIKEFETYKKDILAWINDGRGHEKYTDAKQQLGFIRGGLKGRIKAQKMFRKDKYGKIKSYYENPYTKLTNEFKQISSTYGKTFAELRDKFKEKNNITKITHFGIIIEDNNKDRYLLANGLQHEQINHVEAILGKLNTSSEFITYQVKSLTSKTLIKLIKNHTTKKGAISPYADFHTSKIHVDWTKIKKEWDNYKREQVLLQYVKDCLTDSTMAKNQNWAEFGWNFEKCNSYEDIEHEIDQKSYILQKHTISKQSIASLVEGGCLLLPIINQDITSQGRKDKNQFSKDWKQIFEGSKEFRLHPEFAVSYRTPIKDYPKDKRYGRLQFVCAFNCEIIPQNGEFINLKKQIENFNDEDAQKEAVEEFNKKVNHALLGKEYVVIGIDRGLKQLATLCVLDKRGKILGDFEIYKKEFVRAEKRSKNYWKHTLAETRHILDLSNLRVETTIEDNKVLVDQSLTLVKKNRDTPDEEATEENKQKIKLKQLSYIRKLQHKMQTNEQDVLDLINNEPSDEEFKKRIEGLISSFGEGQKYADLPINTMREMISDLQGVIARGNNQTEKNKIIELDAADNLKQGIVANMIGIVNYIFAKYSYKAYISLEDLSRAYGGAKSGYDGRYLPSTSQDEDVDFKEQQNQMLAGLGTYQFFEMQLLKKLQKIQSDNTVLRFVPAFRSADNYRNIIKLEETKYKSKPFGVVHFIDPKFTSKKCPVCSKTNVYRDKDDILVCKECGFRSDSQLKERENNIHYIHNGDDNGAYHIALKSVENLIQMK

SEQ ID NO: 4 - DNA, 3696 bp, Artificial Sequence
  BEC85 NT Sequence
atgaagtccttcgaaaactcctgccaaatttctaagactttgagattcggtgccactttgaaagaggataagaaaaagtgcaagtcccacttggaattgcaagaattcgttgacatttcctacaagaccttgaagtcatctgctaccattgctgaatccttgaacgaaatcgaattggtcaaaaagtgcgaaaggtgctactccgaaattatcaagttccatgaagcttggggtcaaatctactgtagaactaaccaaattgccgtctacaaggactggtatagacaattggctagaaaggccagattcgatgttggtgatcaaaactctcaactgatcaccttgtcatccttatcttctaagcacaacgtttaccagggtttgaagagatctcaacatattaccaactactggaaggacaacattgccagacaaaagtctttcctgaaggatttctctcaacaattgaagcagtacaagagagctttggaaaattctgataaggctcataccaagccaaacctgattaacttcaacaagaccttctccattttggccaacttggttaacgaaattgtcatcccattgtccaacggtgctatttcttttccaaacatctccaagttggaagatggtgaagaatccagacatttgattgaattcgctctgaacgattactccgatttggttggttctattggtgaattgaaggatgctattgctaccaatggtggttatactccatttgctaaggttaccttgaaccattacactgctgaacaaaagccacacgttttcaagaacgatattgatgccaagatccgtgagttgaagttgattgagttggtcgaaaagttgaagaacaagacgtccaagcaaatcgaagagtacttttccaagttcgacaagttcaagatctacgatgatagaaacatctccgttatcattagaacccaatgctttaagtacaagcccattccatttttggtcaagcacgaattggctaagtatatcgctgaagatgaagatgccgttttgaaggttttggatgcaattggtgctactagatctccagctcatgattacgctcataatgaagatgtttttgacttgaatcactacccaatcaaggttgcttttgattacgcatgggaacaattggctaactccttgtacactactgttactttcccaaaagaacagtgcgagaagtacttgaaggatgtttttgattgcgaagtctccaaagaaccagtttttaagttctacgccgacctgttgtacatcagaaagaatttggctgttttggagcacaagaacaacctgccatctaatcaagaggaattcatctgcaagattaacaacaccttcgagaacatcgttctgccatacaagatttctcaattcgaaacctacaagaaggatatcttggcctggattaacgatggtagaggtcacgaaaagtacaccgatgctaaacaacagttgggttttattagaggtggtctgaaaggtagaatcaaggctcaaaagatgttcagaaaagacaagtacggtaagatcaagtcctactacgaaaacccatacactaagttgaccaacgaattcaagcaaatctcttctacctacggtaaaaccttcgctgaattgagagacaagttcaaagaaaagaacaacatcaccaagatcacccatttcggtattatcatcgaagataagaacagggacagatacttgttggccaacggtttgcaacacgaacaaatcaaccatgtctccaccatcttgaacaagttggataagtcatccgaattcatcacctaccaagttaagtctttgacctctaagaccctgatcaagctgattaagaatcataccaccaagaagggtgcaatttctccatatgctgatttccatacttctaagaccggctttaacaaaaacgagatcgaaaagaactgggacaactacaagagagaacaagtcttggttgaatacgttaaggattgcttgaccgattctaccatggctaagaatcaaaattgggctgaatttggttggaacttcgagaagtgtaactcctacgaagatatcgaacacgaaatcgatcagaagtcttacatcttgcaaaagcataccatttccaagcaatctattgcttctttggttgaaggtggttgtttgttgttgccaattatcaaccaggacatcacctctaaagaacgtaaggacaagaatcagttctccaaggattggaagcaaatcttcgaaggttccaaagaattcagattgcatccagaattcgccgtttcttacagaactccaattgaaggttacccagtccaaaaaagatacggtagattgcaattcgtttgcgcttttaactgcgaaatcatcccacaaaatggtgagttcatcaacttgaagaagcagatcgagaacttcaacgacgaagatgctcaaaaagaagccgtcgaagagttcaacaaaaaggttaaccatgccttgtccgacaaagaatacgttgttattggtatcgacagaggcttgaagcaattagctactttgtgtgttttggacaagaggggtaagattttgggtgactttgaaatctacaaaaaagagttcgtcagagccgaaaagagatctgaatctcattgggaacatactcaagctgaaaccagacatatcttggacttgtctaacttgagagttgaaactaccattgagggcaaaaaggtgttggttgatcaatctttgacactggtcaagaagaacagagatactccagatgaagaagctaccgaagaaaacaagcagaagattaagttgaagcagctgtcctacattagaaagttgcaacacaagatgcagaccaatgaacaagatgtcttggacctgatcaacaacgaaccatctgatgaagaattcaaaaagaggatcgagggcttgatttcttcattcggtgaaggtcaaaagtacgctgatttgcctattaacaccatgagggaaatgatctctgacttgcaaggtgttattgccagaggaaacaatcagactgagaaaaacaagatcatcgaattggatgctgccgacaatttgaaacaaggtatcgttgctaacatgatcggtatcgttaactacattttcgccaagtactcctacaaggcctacatttctttagaagatttgtccagagcttacggtggtgcaaaatctggttatgatggtagatatttgccatccacctctcaagatgaggatgttgactttaaagaacagcagaatcaaatgttggctggcttgggtacttaccaattttttgaaatgcagctgctgaaaaagctgcagaagatccaatctgataacaccgttttgagatttgttccagcttttagatccgccgataactacagaaatatcttgagattggaagagactaagtacaagtctaagccattcggtgttgttcatttcatcgatccaaagttcacatctaagaagtgtccagtttgctctaagactaacgtttacagagataaggatgacatcctggtctgtaaagaatgtggttttaggtccgactcacagttgaaagaaagggaaaacaacatccactacatccacaatggtgatgataatggtgcttaccatattgccttgaagtccgtcgaaaacttgattcagatgaagtaa

SEQ ID NO: 5 - DNA, 3696 bp, Artificial Sequence
  BEC67 NT Sequence
atgaagtccttcgaaaactcctgccaaatttctaagactttgagattcggtgccactttgaaagaggataagaaaaagtgcaagtcccacttggaattgcaagaattcgttgacatttcctacaagaccttgaagtcatctgctaccattgctgaatccttgaacgaaatcgaattggtcaaaaagtgcgaaaggtgctactccgaaattatcaagttccatgaagcttggggtcaaatctactgtagaactaaccaaattgccgtctacaaggactggtatagacaattggctagaaaggccagattcgatgttggtgatcaaaactctcaactgatcaccttgtcatccttatcttctaagcacaacgtttaccagggtttgaagagatctcaacatattaccaactactggaaggacaacattgccagacaaaagtctttcctgaaggatttctctcaacaattgaagcagtacaagagagctttggaaaattctgataaggctcataccaagccaaacctgattaacttcaacaagaccttctccattttggccaacttggttaacgaaattgtcatcccattgtccaacggtgctatttcttttccaaacatctccaagttggaagatggtgaagaatccagacatttgattgaattcgctctgaacgattactccgatttggttggttctattggtgaattgaaggatgctattgctaccaatggtggttatactccatttgctaaggttaccttgaaccattacactgctgaacaaaagccacacgttttcaagaacgatattgatgccaagatccgtgagttgaagttgattgagttggtcgaaaagttgaagaacaagacgtccaagcaaatcgaagagtacttttccaagttcgacaagttcaagatctacgatgatagaaacatctccgttatcattagaacccaatgctttaagtacaagcccattccatttttggtcaagcacgaattggctaagtatatcgctgaagatgaagatgccgttttgaaggttttggatgcaattggtgctactagatctccagctcatgattacgctcataatgaagatgtttttgacttgaatcactacccaatcaaggttgcttttgattacgcatgggaacaattggctaactccttgtacactactgttactttcccaaaagaacagtgcgagaagtacttgaaggatgtttttgattgcgaagtctccaaagaaccagtttttaagttctacgccgacctgttgtacatcagaaagaatttggctgttttggagcacaagaacaacctgccatctaatcaagaggaattcatctgcaagattaacaacaccttcgagaacatcgttctgccatacaagatttctcaattcgaaacctacaagaaggatatcttggcctggattaacgatggtagaggtcacgaaaagtacaccgattctaaaagagaattgggttttattagaggtggtctgaaaggtagaatcaaggctcaaaagatgttcagaaaagacaagtacggtaagatcaagtcctactacgaaaacccatacactaagttgaccgaagagttcaagaacttggccatcacctacggtaaaaccttcgctgaattgagagacaagttcaaagaaaagaacaacatcaccaagatcacccatttcggtattatcatcgaagataagaacagggacagatacttgttggccaacggtttgcaacacgaacaaatcaaccatgtctccaccatcttgaacaagttggataagtcatccgaattcatcacctaccaagttaagtctttgacctctaagaccctgatcaagctgattaagaatcataccaccaagaagggtgcaatttctccatatgctgatttccatacttctaagaccggctttaacaaaaacgagatcgaaaagaactgggacaactacaagagagaacaagtcttggttgaatacgttaaggattgcttgaccgattctaccatggctaagaatcaaaattgggctgaatttggttgggatttggagtcttgtaactcctacgaagatatcgaacacgaaatcgatcagaagtcttacatcttgcaaaagcataccatttccaagcaatctattgcttctttggttgaaggtggttgtttgttgttgccaattatcaaccaggacatcacctctaaagaacgtaaggacaagaatcagttctccaaggattggaagcaaatcttcgaaggttccaaagaattcagattgcatccagaattcgccgtttcttacagaactccaattgaaggttacccagtccaaaaaagatacggtagattgcaattcgtttgcgcttttaactgcgaaatcatcccacaaaatggtgagttcatcaacttgaagaagcagatcgagaacttcaacgacgaagatgctcaaaaagaagccgtcgaagagttcaacaaaaaggttaaccatgccttgtccgacaaagaatacgttgttattggtatcgacagaggcttgaagcaattagctactttgtgtgttttggacaagaggggtaagattttgggtgactttgaaatctacaaaaaagagttcgtcagagccgaaaagagatctgaatctcattgggaacatactcaagctgaaaccagacatatcttggacttgtctaacttgagagttgaaactaccattgagggcaaaaaggtgttggttgatcaatctttgacactggtcaagaagaacagagatactccagatgaagaagctaccgaagaaaacaagcagaagattaagttgaagcagctgtcctacattagaaagttgcaacacaagatgcagaccaatgaacaagatgtcttggacctgatcaacaacgaaccatctgatgaagaattcaaaaagaggatcgagggcttgatttcttcattcggtgaaggtcaaaagtacgctgatttgcctattaacaccatgagggaaatgatctctgacttgcaaggtgttattgccagaggaaacaatcagactgagaaaaacaagatcatcgaattggatgctgccgacaatttgaaacaaggtatcgttgctaacatgatcggtatcgttaactacattttcgccaagtactcctacaaggcctacatttctttagaagatttgtccagagcttacggtggtgcaaaatctggttatgatggtagatatttgccatccacctctcaagatgaggatgttgactttaaagaacagcagaatcaaatgttggctggcttgggtacttaccaattttttgaaatgcagctgctgaaaaagctgcagaagatccaatctgataacaccgttttgagatttgttccagcttttagatccgccgataactacagaaatatcttgagattggaagagactaagtacaagtctaagccattcggtgttgttcatttcatcgatccaaagttcacatctaagaagtgtccagtttgctctaagactaacgtttacagagataaggatgacatcctggtctgtaaagaatgtggttttaggtccgactcacagttgaaagaaagggaaaacaacatccactacatccacaatggtgatgataatggtgcttaccatattgccttgaagtccgtcgaaaacttgattcagatgaagtaa

SEQ ID NO: 6 - DNA, 3696 bp, Artificial Sequence
  BEC10 NT Sequence
atgaagtccttcgaaaactcctgccaaatttctaagactttgagattcggtgccactttgaaagaggataagaaaaagtgcaagtcccacttggaattgcaagaattcgttgacatttcctacaagaccttgaagtcatctgctaccattgctgaatccttgaacgaaatcgaattggtcaaaaagtgcgaaaggtgctactccgaaattatcaagttccatgaagcttggggtcaaatctactgtagaactaaccaaattgccgtctacaaggactggtatagacaattggctagaaaggccagattcgatgttggtgatcaaaactctcaactgatcaccttgtcatccttatcttctaagcacaacgtttaccagggtttgaagagatctcaacatattaccaactactggaaggacaacattgccagacaaaagtctttcctgaaggatttctctcaacaattgaagcagtacaagagagctttggaaaattctgataaggctcataccaagccaaacctgattaacttcaacaagaccttctccattttggccaacttggttaacgaaattgtcatcccattgtccaacggtgctatttcttttccaaacatctccaagttggaagatggtgaagaatccagacatttgattgaattcgctctgaacgattactccgatttggttggttctattggtgaattgaaggatgctattgctaccaatggtggttatactccatttgctaaggttaccttgaaccattacactgctgaacaaaagccacacgttttcaagaacgatattgatgccaagatccgtgagttgaagttgattgagttggtcgaaaagttgaagaacaagacgtccaagcaaatcgaagagtacttttccaagttcgacaagttcaagatctacgatgatagaaacatctccgttatcattagaacccaatgctttaagtacaagcccattccatttttggtcaagcacgaattggctaagtatatcgctgaagatgaagatgccgttttgaaggttttggatgcaattggtgctactagatctccagctcatgattacgctcataatgaagatgtttttgacttgaatcactacccaatcaaggttgcttttgattacgcatgggaacaattggctaacggtgtctacactactgttactttcccaaaagaacagtgcgagaagtacttgaaggatgtttttgattgcgaagtctccaaagaaccagtttttaagttctacgccgacctgttgtacatcagaaagaatttggctgttttggagcacaagaacaacctgccatctaatcaagaggaattcatctgcaagattaacaacaccttcgagaacatcgttctgccatacaagattaaagagttcgaaacctacaagaaggatatcttggcctggattaacgatggtagaggtcacgaaaagtacaccgatgctaaacaacagttgggttttattagaggtggtctgaaaggtagaatcaaggctcaaaagatgttcagaaaagacaagtacggtaagatcaagtcctactacgaaaacccatacactaagttgaccaacgaattcaagcaaatctcttctacctacggtaaaaccttcgctgaattgagagacaagttcaaagaaaagaacaacatcaccaagatcacccatttcggtattatcatcgaagataacaacaaagacagatacttgttggccaacggtttgcaacacgaacaaatcaaccatgtcgaagccattttgggtaagttgaacacctcatccgaattcatcacctaccaagttaagtctttgacctctaagaccctgatcaagctgattaagaatcataccaccaagaagggtgcaatttctccatatgctgatttccatacttctaagatccatgttgattggaccaagatcaagaaagaatgggacaactacaagagagaacaagtcttgttgcaatacgttaaggattgcttgaccgattctaccatggctaagaatcaaaattgggctgaatttggttggaacttcgagaagtgtaactcctacgaagatatcgaacacgaaatcgatcagaagtcttacatcttgcaaaagcataccatttccaagcaatctattgcttctttggttgaaggtggttgtttgttgttgccaattatcaaccaggacatcacctctcaaggtcgtaaggacaagaatcagttctccaaggattggaagcaaatcttcgaaggttccaaagaattcagattgcatccagaattcgccgtttcttacagaactccaattaaggactacccaaaggataaaagatacggtagattgcaattcgtttgcgcttttaactgcgaaatcatcccacaaaatggtgagttcatcaacttgaagaagcagatcgagaacttcaacgacgaagatgctcaaaaagaagccgtcgaagagttcaacaaaaaggttaaccatgccttgttgggtaaagaatacgttgttattggtatcgacagaggcttgaagcaattagctactttgtgtgttttggacaagaggggtaagattttgggtgactttgaaatctacaaaaaagagttcgtcagagccgaaaagagatctaagaattactggaagcacaccttggctgaaaccagacatatcttggacttgtctaacttgagagttgaaactaccattgaggataataaggtgttggttgatcaatctttgacactggtcaagaagaacagagatactccagatgaagaagctaccgaagaaaacaagcagaagattaagttgaagcagctgtcctacattagaaagttgcaacacaagatgcagaccaatgaacaagatgtcttggacctgatcaacaacgaaccatctgatgaagaattcaaaaagaggatcgagggcttgatttcttcattcggtgaaggtcaaaagtacgctgatttgcctattaacaccatgagggaaatgatctctgacttgcaaggtgttattgccagaggaaacaatcagactgagaaaaacaagatcatcgaattggatgctgccgacaatttgaaacaaggtatcgttgctaacatgatcggtatcgttaactacattttcgccaagtactcctacaaggcctacatttctttagaagatttgtccagagcttacggtggtgcaaaatctggttatgatggtagatatttgccatccacctctcaagatgaggatgttgactttaaagaacagcagaatcaaatgttggctggcttgggtacttaccaattttttgaaatgcagctgctgaaaaagctgcagaagatccaatctgataacaccgttttgagatttgttccagcttttagatccgccgataactacagaaatatcatcaagttggaagagactaagtacaagtctaagccattcggtgttgttcatttcatcgatccaaagttcacatctaagaagtgtccagtttgctctaagactaacgtttacagagataaggatgacatcctggtctgtaaagaatgtggttttaggtccgactcacagttgaaagaaagggaaaacaacatccactacatccacaatggtgatgataatggtgcttaccatattgccttgaagtccgtcgaaaacttgattcagatgaagtaa

SEQ ID NO: 7 - DNA, 19 bp, Artificial Sequence
  BEC Family gRNA Sequence
gatttctactattgtagat

SEQ ID NO: 8 - DNA, 19 bp, Artificial Sequence
  BEC Family gRNA Sequence (consensus)
  variation 1,11: /replace="a,c,g,t"
natttctactnttgtagat

SEQ ID NO: 9 - DNA, 68 bp, Artificial Sequence
  HDV Self-Splicing Sequence
ggccggcatggtcccagcctcctcgctggcgccggctgggcaacatgcttcggcatggcgaatgggac

SEQ ID NO: 10 - DNA, 43 bp, Artificial Sequence
  Hammerhead Ribozyme (HH) Self-Splicing Sequence
gaaattctgatgagtccgtgaggacgaaacgagtaagctcgtc

SEQ ID NO: 11 - DNA, 886 bp, Artificial Sequence
  Tef1 Promoter Sequence
cgagacagcagaatcaccgcccaagttaagcctttgtgctgatcatgctctcgaacgggccaagttcgggaaaagcaaaggagcgtttagtgaggggcaatttgactcacctcccaggcaacagatgaggggggcaaaaagaaagaaattttcgtgagtcaatatggattccgagcatcattttcttgcggtctatcttgctacgtatgttgatcttgacgctgtggatcaagcaacgccactcgctcgctccatcgcaggctggtcgcagacaaattaaaaggcggcaaactcgtacagccgcggggttgtccgctgcaaagtacagagtgataaaagccgccatgcgaccatcaacgcgttgatgcccagctttttcgatccgagaatccaccgtagaggcgatagcaagtaaagaaaagctaaacaaaaaaaaatttctgcccctaagccatgaaaacgagatggggtggagcagaaccaaggaaagagtcgcgctgggctgccgttccggaaggtgttgtaaaggctcgacgcccaaggtgggagtctaggagaagaatttgcatcgggagtggggcgggttacccctccatatccaatgacagatatctaccagccaagggtttgagcccgcccgcttagtcgtcgtcctcgcttgcccctccataaaaggatttcccctccccctcccacaaaattttctttcccttcctctccttgtccgcttcagtacgtatatcttcccttccctcgcttctctcctccatccttctttcatccatctcctgctaacttctctgctcagcacctctacgcattactagccgtagtatctgagcacttctcccttttatattccacaaaacataacacaaccttcacc

SEQ ID NO: 12 - DNA, 235 bp, Artificial Sequence
  TtrpC Terminator Sequence
tgatttaatagctccatgtcaacaagaataaaacgcgtttcgggtttacctcttccagatacagctcatctgcaatgcattaatgcattggacctcgcaaccctagtacgcccttcaggctccggcgaagcagaagaatagcttagcagagtctattttcattttcgggagacgagatcaagcagatcaacggtcgtcaagagacctacgagactgaggaatccgctcttggctc

SEQ ID NO: 13 - protein, 9 aa, Artificial Sequence
  C-myc NLS
PAAKKKKLD

SEQ ID NO: 14 - protein, 16 aa, Artificial Sequence
  Neoplasmin NLS
KRPAATKKAGQAKKKK

SEQ ID NO: 15 - protein, 7 aa, Artificial Sequence
  SV40 NLS
PKKKRKV

SEQ ID NO: 16 - DNA, 3816 bp, Artificial Sequence
  BEC10 NT Sequence Codon optimized for Aspergillus Niger
atgaagtccttcgagaactcctgccagatcagcaagaccctccgcttcggcgctaccctcaaagaggataagaagaagtgcaagtcccacctcgagctgcaagagttcgtcgatatctcctacaagaccctgaagtcctccgccactatcgctgagtccctcaacgagatcgagctggtcaagaagtgcgagcgctgctactccgagatcatcaagttccacgaggcttggggccagatctactgccgcaccaaccagatcgccgtctacaaggattggtatcgccagctcgcccgcaaggcccgcttcgatgtcggcgatcagaactcccagctcattaccctctccagcctgtcctccaagcacaacgtctaccagggcctcaagcgctcccagcacatcaccaactactggaaggataatatcgcccgccagaagtcgttcctcaaggatttctcccagcagctcaagcagtacaagcgcgccctcgagaacagcgataaggcccacaccaagcctaacctcatcaacttcaacaagaccttctccatcctcgccaacctcgtcaacgaaatcgtcatccctctctccaacggcgccatcagcttccccaacatctccaagctcgaggacggcgaggaatcccgccacctcatcgagttcgccctgaacgattactccgatctcgtcggctccatcggcgagctgaaggatgctatcgccaccaacggcggctacacccctttcgccaaggtcactctcaaccactacaccgccgagcagaagccccacgttttcaagaacgatatcgatgccaagatccgcgagttgaagctcatcgaactcgtcgagaagctcaagaacaagaccagcaagcagatcgaggaatacttctccaagttcgataagttcaagatctacgatgatcgcaacatcagcgtcatcatccgcactcagtgcttcaagtacaagcccattccgttcctcgtcaagcacgagctggccaagtatatcgccgaggatgaggatgccgtcctcaaggtcctcgatgccatcggcgccactcgctccccggctcacgattacgcccacaacgaggatgtgttcgatctcaatcactaccccatcaaggtcgccttcgactacgcctgggagcagctcgccaacggtgtctacaccaccgtcactttccccaaagagcagtgcgagaagtacctcaaggacgtgttcgactgcgaggtgtccaaagaacccgtgttcaagttctatgccgatctcctctacatccgcaagaacctggccgtcctggaacacaagaacaacctgccttccaatcaagaggaattcatctgcaagatcaacaacacgttcgagaacatcgtcctgccttacaagatcaaagagttcgaaacctacaagaaggacatcctggcctggatcaacgatggccgcggtcatgagaagtacaccgacgccaagcagcagctcggcttcatccgcggtggcctcaagggccgcatcaaggcccagaagatgttccggaaggacaagtacggtaagatcaagtcctactacgagaacccctacaccaagctcaccaacgagttcaagcaaatctcctccacctacggaaagaccttcgctgagctgcgcgacaagttcaaagaaaagaacaatatcaccaagatcacccacttcggcatcatcatcgaggataacaacaaggatcgctacctcctggccaacggcctccagcacgagcagatcaaccacgtcgaggccatcctgggcaagctcaacacctccagcgagttcatcacctaccaggtcaagtccctcacctccaagactctcatcaagctgatcaagaaccacaccaccaagaagggcgccatctcgccctacgccgatttccataccagcaagatccacgtcgattggaccaagattaagaaagagtgggataactataagcgcgagcaggtcctcctgcagtacgtcaaggattgcctcaccgattccaccatggccaagaaccagaactgggccgagttcggctggaacttcgaaaagtgcaactcctacgaggatatcgagcatgagatcgatcagaagtcctacatcctccagaagcacaccatctcgaagcagtcgatcgcttccctggtggaaggcggctgcctgctgctccccatcatcaaccaggatatcaccagccagggccgcaaggacaagaatcagttcagcaaggactggaagcagatcttcgagggctcgaaagagttccgcctccatcctgagttcgccgtgtcctatcgcacccctatcaaggattaccccaaggataagcgctacggccgcctccagttcgtctgcgccttcaactgcgagatcattccccagaacggcgaattcatcaacctcaagaagcaaatcgagaacttcaacgatgaggacgcccagaaagaggccgtcgaagagtttaacaagaaggtcaaccacgctctcctcggcaaagagtatgtcgtcatcggcatcgatcgcggcctgaagcagctggctaccctctgcgtcctcgataagcgcggcaagatcctgggcgatttcgagatctacaagaaagaattcgtccgcgccgagaagcgctccaagaactattggaagcacactctcgccgagactcgccacatcctggatctgtccaacctccgcgtcgaaaccaccattgaggacaacaaggtcctggtcgatcagtcgctcaccctcgtgaagaagaaccgcgatacccctgatgaggaagccaccgaggaaaacaagcagaagattaagctgaagcaactgtcctatatccgcaagctccagcacaagatgcagaccaacgagcaggatgtgctcgacctgatcaacaatgagccctccgatgaagagttcaagaagcggatcgagggcctcatctcctcgttcggcgagggccagaagtacgccgatctgcccatcaacaccatgcgcgagatgatctccgatctgcagggcgtgatcgctcgcggcaacaaccagaccgagaagaacaaaatcattgagctggatgccgccgataacctcaagcagggcatcgtcgccaacatgatcggtatcgtcaactacatcttcgccaagtacagctacaaggcttacatctccctcgaggatctctcccgcgcctacggcggtgccaagtccggctacgacggccgctacctgccgtcgacctcgcaggacgaggacgtcgatttcaaagaacagcagaaccagatgctcgccggcctcggcacctatcagttcttcgaaatgcagctcctgaagaagctccagaagatccagtccgataacaccgtcctgcgcttcgtccccgccttccgctccgccgacaactaccgcaacattatcaagctcgaagagactaagtacaagtccaagcctttcggcgtcgtccacttcatcgatcccaagttcacctctaagaagtgccccgtctgctccaagaccaacgtgtaccgcgataaggatgatattctcgtctgcaaagagtgcggcttccgcagcgattcccagctgaaagagcgcgagaacaacatccactacatccacaacggcgacgataacggcgcctaccatatcgccctcaagtcggtcgagaacctcatccagatgaagaagcgcccagccgccactaagaaggccggccaggctaagaagaaaaaggcctccggctccggcgctggctcccctaagaaaaagcgcaaggtcgaggatcccaaaaagaagcgtaaggtctga

SEQ ID NO: 17 - DNA, 5749 bp, Artificial Sequence
  Fungal AMA1 autonomously replicating sequence
ccgggcccagtatatgttccgcagatgactggagctctgccatacgtgccctctcaagcaccatttgttccatctacagagactagtcaccaactagtctatcaagactcacagggtacattgctgagaccaactgaccagaggcagggtagcggattgacggctccatctccttcacttacaaggtctattgaaagccctttagcatcaccaagcggagaatagattgttaagcttattttttgtatactgttttgtgatagcacgaagtttttccacggtatcttgtaaaaatatatatttgtggcgggcttacctacatcaaattaataagagactaattataaactaaacacacaagcaagctactttagggtaaaagtttataaatgcttttgacgtataaacgttgcttgtatttattattacaattaaaggtggatagaaaacctagagactagttagaaactaatctcaggtttgcgttaaactaaatcagagcccgagaggttaacagaacctagaaggggactagatatccgggtagggaaacaaaaaaaaaaaacaagacagccacatattagggagactagttagaagctagttccaggactaggaaaataaaagacaatgataccacagtctagttgacaactagatagattctagattgaggccaaagtctctgagatccaggttagttgcaactaatactagttagtatctagtctcctataactctgaagctagaataacttactactattatcctcaccactgttcagctgcgcaaacggagtgattgcaaggtgttcagagactagttattgactagtcagtgactagcaataactaacaaggtattaacctaccatgtctgccatcaccctgcacttcctcgggctcagcagccttttcctcctcattttcatgctcattttccttgtttaagactgtgactagtcaaagactagtccagaaccacaaaggagaaatgtcttaccactttcttcattgcttgtctcttttgcattatccatgtctgcaactagttagagtctagttagtgactagtccgacgaggacttgcttgtctccggattgttggaggaactctccagggcctcaagatccacaacagagccttctagaagactggtcaataactagttggtctttgtctgagtctgacttacgaggttgcatactcgctccctttgcctcgtcaatcgatgagaaaaagcgccaaaactcgcaatatggctttgaaccacacggtgctgagactagttagaatctagtcccaaactagcttggatagcttacctttgccctttgcgttgcgacaggtcttgcagggtatggttcctttctcaccagctgatttagctgccttgctaccctcacggcggatctgccataaagagtggctagaggttataaattagcactgatcctaggtacggggctgaatgtaacttgcctttcctttctcatcgcgcggcaagacaggcttgctcaaattcctaccagtcacaggggtatgcacggcgtacggaccacttgaactagtcacagattagttagcaactagtctgcattgaatggctgtacttacgggccctcgccattgtcctgatcatttccagcttcaccctcgttgctgcaaagtagttagtgactagtcaaggactagttgaaatgggagaagaaactcacgaattctcgactcccttagtattgtggtccttggacttggtgctgctatatattagctaatacactagttagactcacagaaacttacgcagctcgcttgcgcttcttggtaggagtcggggttgggagaacagtgccttcaaacaagccttcataccatgctacttgactagtcagggactagtcaccaagtaatctagataggacttgcctttggcctccatcagttccttcatagtgggaggaccattgtgcaatgtaaactccatgccgtgggagttcttgtccttcaagtgcttgaccaatatgtttctgttggcagagggaacctgtcaactagttaataactagtcagaaactatgatagcagtagactcactgtacgcttgaggcatcccttcactcggcagtagacttcatatggatggatatcaggcacgccattgtcgtcctgtggactagtcagtaactaggcttaaagctagtcgggtcggcttactatcttgaaatccggcagcgtaagctccccgtccttaactgcctcgagatagtgacagtactctggggactttcggagatcgttatcgttatcgcgaatgctcggcatactaactgttgactagtcttggactagtcccgagcaaaaaggattggaggaggaggaggaaggtgagagtgagacaaagagcgaaataagagcttcaaaggctatctctaagcagtatgaaggttaagtatctagttcttgactagatttaaagagatttcgactagttatgtacctggagtttggatataggaatgtgttgtggtaacgaaatgtaagggggaggaaagaaaaagtcgtcaagaggtaactctaagtcggccattcctttttgggaggcgctaaccataaacggcatggtcgacttagagttagctcagggaatttagggagttatctgcgaccaccgaggaacggcggaatgccaaagaatcccgatggagctctagctggcggttgacaaccccaccttttggcgtttctgcggcgttgcaggcgggactggatacttcgtagaaccagaaaggcaaggcagaacgcgctcagcaagagtgttggaagtgatagcatgatgtgccttgttaactaggtaccaatctgcagtatgcttgatgttatccaaagtgtgagagaggaaggtccaaacatacacgattgggagagggcctaggtataagagtttttgagtagaacgcatgtgagcccagccatctcgaggagattaaacacgggccggcatttgatggctatgttagtaccccaatggaaacggtgagagtccagtggtcgcagataactccctaaattccctgagctaactctaagtcgaccatgccgtttatggttagcgcctcccaaaaaggaatggccgacttagagttacctcttgacgactttttctttcctcccccttacatttcgttaccacaacacattcctatatccaaactccaggtacataactagtcgaaatctctttaaatctagtcaagaactagatacttaaccttcatactgcttagagatagcctttgaagctcttatttcgctctttgtctcactctcaccttcctcctcctcctccaatcctttttgctcgggactagtccaagactagtcaacagttagtatgccgagcattcgcgataacgataacgatctccgaaagtccccagagtactgtcactatctcgaggcagttaaggacggggagcttacgctgccggatttcaagatagtaagccgacccgactagctttaagcctagttactgactagtccacaggacgacaatggcgtgcctgatatccatccatatgaagtctactgccgagtgaagggatgcctcaagcgtacagtgagtctactgctatcatagtttctgactagttattaactagttgacaggttccctctgccaacagaaacatattggtcaagcacttgaaggacaagaactcccacggcatggagtttacattgcacaatggtcctcccactatgaaggaactgatggaggccaaaggcaagtcctatctagattacttggtgactagtccctgactagtcaagtagcatggtatgaaggcttgtttgaaggcactgttctcccaaccccgactcctaccaagaagcgcaagcgagctgcgtaagtttctgtgagtctaactagtgtattagctaatatatagcagcaccaagtccaaggaccacaatactaagggagtcgagaattcgtgagtttcttctcccatttcaactagtccttgactagtcactaactactttgcagcaacgagggtgaagctggaaatgatcaggacaatggcgagggcccgtaagtacagccattcaatgcagactagttgctaactaatctgtgactagttcaagtggtccgtacgccgtgcatacccctgtgactggtaggaatttgagcaagcctgtcttgccgcgcgatgagaaaggaaaggcaagttacattcagccccgtacctaggatcagtgctaatttataacctctagccactctttatggcagatccgccgtgagggtagcaaggcagctaaatcagctggtgagaaaggaaccataccctgcaagacctgtcgcaacgcaaagggcaaaggtaagctatccaagctagtttgggactagattctaactagtctcagcaccgtgtggttcaaagccatattgcgagttttggcgctttttctcatcgattgacgaggcaaagggagcgagtatgcaacctcgtaagtcagactcagacaaagaccaactagttattgaccagtcttctagaaggctctgttgtggatcttgaggccctggagagttcctccaacaatccggagacaagcaagtcctcgtcggactagtcactaactagactctaactagttgcagacatggataatgcaaaagagacaagcaatgaagaaagtggtaagacatttctcctttgtggttctggactagtctttgactagtcacagtcttaaacaaggaaaatgagcatgaaaatgaggaggaaaaggctgctgagcccgaggaagtgcagggtgatggcagacatggtaggttaataccttgttagttattgctagtcactgactagtcaataactagtctctgaacaccttgcaatcactccgtttgcgcagctgaacagtggtgaggataatagtagtaagttattctagcttcagagttataggagactagatactaactagtattagttgcaactaacctggatctcagagactttggcctcaatctagaatctatctagttgtcaactagactgtggtatcattgtcttttattttcctagtcctggaactagcttctaactagtctccctaatatgtggctgtcttgttttttttttttgtttccctacccggatatctagtccccttctaggttctgttaacctctcgggctctgatttagtttaacgcaaacctgagattagtttctaactagtctctaggttttctatccacctttaattgtaataataaatacaagcaacgtttatacgtcaaaagcatttataaacttttaccctaaagtagcttgcttgtgtgtttagtttataattagtctcttattaatttgatgtaggtaagcccgccacaaatatatatttttacaagataccgtggaaaaacttcgtgctatcacaaaacagtatacaaaaaataagcttaacaatctattctccgcttggtgatgctaaagggctttcaatagaccttgtaagtgaaggagatggagccgtcaatccgctaccctgcctctggtcagttggtctcagcaatgtaccctgtgagtcttgatagactagttggtgactagtctctgtagatggaacaaatggtgcttgagagggcacgtatggcagagctccagtcatctgcggaacatatactgggcccgggaagatctcatggtcatagctgtttccg

SEQ ID NO: 18 - DNA, 24 bp, Artificial Sequence
  Ku70 Specific 24 bps Target Sequence
gaatcagattgtagatatgcaggc

SEQ ID NO: 19 - DNA, 489 bp, Artificial Sequence
  Tef1 Terminator Sequence
gcggacattcgatttatgccgttatgacttccttaaaaaagcctttacgaatgaaagaaatggaattagacttgttatgtagttgattctacaatggattatgattcctgaacttcaaatccgctgttcattattaatctcagttcttcccgtaaagccaatgttgaaactattcgtaaatgtacctcgttttgcgtgtaccttgcttatcacgtgatattacatgacctggacagagttctgcgcgaaagtcataacgtaaatcccgggcggtaggtgcgtcccgggcggaaggtagttttctcgtccaccccaacgcgtttatcaacctcaactttcaacaaccatcatgccaccaaaagcgcgtaaaacaaagcgagatttgattgagcaagagggcaggatccaatgcgcgattcaagacattaaaaatggaaaatttcaaaaaattgcgcccgcagcgcgtgcatacaaaattcatcccaatac

SEQ ID NO: 20 - DNA, 497 bp, Artificial Sequence
  PgpdA Promoter from A. Nidulans
gcgtaagctccctaattggcccatccggcatctgtagggcgtccaaatatcgtgcctctcctgctttgcccggtgtatgaaaccggaaaggccgctcaggagctggccagcggcgcagaccgggaacacaagctggcagtcgacccatccggtgctctgcactcgacctgctgaggtccctcagtccctggtaggcagctttgccccgtctgtccgcccggtgtgtcggcggggttgacaaggtcgttgcgtcagtccaacatttgttgccatattttcctgctctccccaccagctgctcttttcttttctctttcttttcccatcttcagtatattcatcttcccatccaagaacctttatttcccctaagtaagtactttgctacatccatactccatccttcccatcccttattcctttgaacctttcagttcgagctttcccacttcatcgcagcttgactaacagctaccccgcttgagcagacatcaccg

SEQ ID NO: 21 - DNA, 2233 bp, Artificial Sequence
  HDR template
ttcggttgacctagtcaatggaggtaataagaaaagaccgttcgtatcgcgcaagcagatgaactattcacgccgcattaaatattcaaaagatggacgagtggcaagaacaggtagtgggtgtatacaacagcgcaaggccttctggaagctgaaaagtccagaacggcttgatgacggagcaccgagaccacgaccaactccgactcccgacagccaatgaccggccagctagcgtcatcaattaccgggcggacatcacatgatgttcgtgtctccccgcgtctttctgcccaccggtttgatcgcgtccctcgcgaccggatccagtgacgatatagatagatctatctccggctgcaggcagcagaggccaaacaggcagacacaacagccccacttgttcctggttacgattcaagttgtcttaacctttatacttccctctttcaatttcgataatatcttgaatgctttaaacgattccacaacattctactgacctgcgttatagcttcccgttagttatagtaccatcgttataccagccaatcaagtcaccacgcacgaccggggacggcgaatccccgggaattgaaagaaattgcatcccaggccagtgaggccagcgattggccacctctccaaggcacagggccattctgcagcgctggtggattcatcgcaatttcccccggcccggcccgacaccgctataggctggttctcccacaccatcggagattcgtcgcctaatgtctcgtccgttcacaagctgaagagcttgaagtggcgagatgtctctgcaggaattcaagctagatgctaagcgatattgcatggcaatatgtgttgatgcatgtgcttcttccttcagcttcccctcgtgcagatgaggtttggctataaattgaagtggttggtcggggttccgtgaggggctgaagtgcttcctcccttttagacgcaactgagagcctgagcttcatccccagcatcattacacctcagcaatggtgagcaagggcgaggagctgttcaccggggtggtgcccatcctggtcgagctggacggcgacgtaaacggccacaagttcagcgtgtccggcgagggcgagggcgatgccacctacggcaagctgaccctgaagttcatctgcaccaccggcaagctgcccgtgccctggcccaccctcgtgaccaccttcacctacggcgtgcagtgcttcagccgctaccccgaccacatgaagcagcacgacttcttcaagtccgccatgcccgaaggctacgtccaggagcgcaccatcttcttcaaggacgacggcaactacaagacccgcgccgaggtgaagttcgagggcgacaccctggtgaaccgcatcgagctgaagggcatcgacttcaaggaggacggcaacatcctggggcacaagctggagtacaactacaacagccacaacgtctatatcatggccgacaagcagaagaacggcatcaaggtgaacttcaagatccgccacaacatcgaggacggcagcgtgcagctcgccgaccactaccagcagaacacccccatcggcgacggccccgtgctgctgcccgacaaccactacctgagcacccagtccgccctgagcaaagaccccaacgagaagcgcgatcacatggtcctgctggagttcgtgaccgccgccgggatcactctcggcatggacgagctgtacaagtgacatggcgggattgttggattcgctagtgcgcttctgttggtggatgtcgttatgtggtgtcttatctcgggttaggcgttcgtgacctgaggacatgagcttgtaattaatgatgggttggatgtcgcggtattcgttcttcagcgaaacgtaatggacacgtattttaggcgatgtacagttataaaaaatcgaattcgctgggctagccggacatgtcaaaacgaagagcattaggagagacatatcaggtccaagtgctatctttcaaaccagtcgcttaagatcaccgaggcatttatctccagaaaattcaccggttcagcaggtgcgcgtatcccgaattcaaattaatattggaacgatcgtaaataaccacccagattcgccgtaaacgatagtagtcaggctttgccgccgacagaaggggacgagtatgtcaactgagtcaacttgaaccgagcagtccctgtaaacaacgccacgctgtttgtaatatc